European Patent Application EP 4 378 925 A1, published June 5, 2024. Title: UNNATURAL AMINO ACID AND USE THEREOF, RECOMBINANT PROTEIN CONTAINING SAME AND RECOMBINANT PROTEIN CONJUGATE. Applicant: Novocodex Biopharmaceuticals Co., Ltd. Application PCT/CN2021/109277. The sequence listing filed with the application follows.

SEQUENCE LISTING (7 sequences)

SEQ ID NO: 1 - protein, 191 aa, Homo sapiens [sequence omitted]

SEQ ID NO: 2 - DNA, 603 bp, Artificial sequence
  Recombinant human growth hormone
atgtttcctactataccactatctcgtctattcgataacgctatgcttcgggcccatcgtcttcatcagctggcctttgacacctaccaggagtttgaagaagcctatatcccaaaggaacagaagtattcattcctgcagaacccccagacctccctctgtttctcagagtctattccgacaccctccaacagggaggaaacacaacagaaatccaacctagagctgctccgcatctccctgctgctcatccagtcgtggctggagcccgtgcagttcctcaggagtgtcttcgccaacagcctggtgtacggcgcctcttagagcaacgtctatgacctcctaaaggacctagaggaaggcatccaaacgctgatggggaggctggaagatggcagcccccggactgggcagatcttcaagcagacctacagcaagttcgacacaaactcacacaacgatgacgcactactcaagaactacgggctgctctactgcttcaggaaggacatggacaaggtcgagacattcctgcgcatcgtgcagtgccgctctgtggagggcagctgtggcttcctcgagcaccaccaccaccaccactaa

SEQ ID NO: 3 - DNA, 753 bp, Artificial sequence
  Wild-type green fluorescent protein containing the purification tag
atggtgagcaagggcgaggagctgttcaccggggtggtgcccatcctggtcgagctggacggcgacgtaaacggccacaagttcagcgtgtccggcgagggcgagggcgatgccacctagggcaagctgaccctgaagttcatctgcaccaccggcaagctgcccgtgccctggcccaccctcgtgaccaccctgacctacggcgtgcagtgcttcagccgctaccccgaccacatgaagcagcacgacttcttcaagtccgccatgcccgaaggctacgtccaggagcgcaccatcttcttcaaggacgacggcaactacaagacccgcgccgaggtgaagttcgagggcgacaccctggtgaaccgcatcgagctgaagggcatcgacttcaaggaggacggcaacatcctggggcacaagctggagtacaactacaacagccacaacgtctatatcatggccgacaagcagaagaacggcatcaaggtgaacttcaagatccgccacaacatcgaggacggcagcgtgcagctcgccgaccactaccagcagaacacccccatcggcgacggccccgtgctgctgcccgacaaccactacctgagcacccagtccgccctgagcaaagaccccaacgagaagcgcgatcacatggtcctgctggagttcgtgaccgccgccgggatcactctcggcatggacgagctgtacaagaagtacgaagattacaaggatgacgacgataagtaa

SEQ ID NO: 4 - DNA, 6170 bp, Artificial sequence
  Expression plasmid pEGFP40
gttaggcgttttgcgctgcttcgcgatgtacgggccagatatacgcgttgacattgattattgactagttattaatagtaatcaattacggggtcattagttcatagcccatatatggagttccgcgttacataacttacggtaaatggcccgcctggctgaccgcccaacgacccccgcccattgacgtcaataatgacgtatgttcccatagtaacgccaatagggactttccattgacgtcaatgggtggagtatttacggtaaactgcccacttggcagtacatcaagtgtatcatatgccaagtacgccccctattgacgtcaatgacggtaaatggcccgcctggcattatgcccagtacatgaccttatgggactttcctacttggcagtacatctacgtattagtcatcgctattaccatggtgatgcggttttggcagtacatcaatgggcgtggatagcggtttgactcacggggatttccaagtctccaccccattgacgtcaatgggagtttgttttggcaccaaaatcaacgggactttccaaaatgtcgtaacaactccgccccattgacgcaaatgggcggtaggcgtgtacggtgggaggtctatataagcagagctcgtttagtgaaccgtcagatcgcctggagacgccatccacgctgttttgacctccatagaagacaccgggaccgatccagcctccggactctagaggatccccgccaccatggtgagcaagggcgaggagctgttcaccggggtggtgcccatcctggtcgagctggacggcgacgtaaacggccacaagttcagcgtgtccggcgagggcgagggcgatgccacctagggcaagctgaccctgaagttcatctgcaccaccggcaagctgcccgtgccctggcccaccctcgtgaccaccctgacctacggcgtgcagtgcttcagccgctaccccgaccacatgaagcagcacgacttcttcaagtccgccatgcccgaaggctacgtccaggagcgcaccatcttcttcaaggacgacggcaactacaagacccgcgccgaggtgaagttcgagggcgacaccctggtgaaccgcatcgagctgaagggcatcgacttcaaggaggacggcaacatcctggggcacaagctggagtacaactacaacagccacaacgtctatatcatggccgacaagcagaagaacggcatcaaggtgaacttcaagatccgccacaacatcgaggacggcagcgtgcagctcgccgaccactaccagcagaacacccccatcggcgacggccccgtgctgctgcccgacaaccactacctgagcacccagtccgccctgagcaaagaccccaacgagaagcgcgatcacatggtcctgctggagttcgtgaccgccgccgggatcactctcggcatggacgagctgtacaagaagtacgaagattacaaggatgacgacgataagtaagaattccggaagggttcgatccctaccggttagtaatgagtttaaacgggggaggctaactgaaacacggaaggagacaataccggaaggaacccgcgctatgacggcaataaaaagacagaataaaacgcacgggtgttgggtcgtttgttcataaacgcggggttcggtcccagggctggcactctgtcgataccccaccgagaccccattggggccaatacgcccgcgtttcttccttttccccaccccaccccccaagttcgggtgaaggcccagggctcgcagccaacgtcggggcggcaggccctgccatagcagatctgcgcagctggggctctagggggtatccccacgcgccctgtagcggcgcattaagcgcggcgggtgtggtggttacgcgcagcgtgaccgctacacttgccagcgccctagcgcccgctcctttcgctttcttcccttcctttctcgccacgttcgccggctttccccgtcaagctctaaatcggggcatccctttagggttccgatttagtgctttacggcacctcgaccccaaaaaacttgattagggtgatggttcacgtagtgggccatcgccctgatagacggtttttcgccctttgacgttggagtccacgttctttaatagtggactcttgttccaaactggaacaacactcaaccctatctcggtctattcttttgatttataagggattttggggatttcggcctattggttaaaaaatgagctgatttaacaaaaatttaacgcgaattaattctgtggaatgtgtgtcagttagggtgtggaaagtccccaggctccccagcaggcagaagtatgcaaagcatgcatctcaattagtcagcaaccaggtgtggaaagtccccaggctccccagcaggcagaagtatgcaaagcatgcatctcaattagtcagcaaccatagtcccgcccctaactccgcccatcccgcccctaactccgcccagttccgcccattctccgccccatggctgactaattttttttatttatgcagaggccgaggccgcctctgcctctgagctattccagaagtagtgaggaggcttttttggaggcctaggcttttgcaaaaagctcccgggagcttgtatatccattttcggatctgatcaagagacaggatgaggatcgtttcgcatgattgaacaagatggattgcacgcaggttctccggccgcttgggtggagaggctattcggctatgactgggcacaacagacaatcggctgctctgatgccgccgtgttccggctgtcagcgcaggggcgcccggttctttttgtcaagaccgacctgtccggtgccctgaatgaactgcaggacgaggcagcgcggctatcgtggctggccacgacgggcgttccttgcgcagctgtgctcgacgttgtcactgaagcgggaagggactggctgctattgggcgaagtgccggggcaggatctcctgtcatctcaccttgctcctgccgagaaagtatccatcatggctgatgcaatgcggcggctgcatacgcttgatccggctacctgcccattcgaccaccaagcgaaacatcgcatcgagcgagcacgtactcggatggaagccggtcttgtcgatcaggatgatctggacgaagagcatcaggggctcgcgccagccgaactgttcgccaggctcaaggcgcgcatgcccgacggcgaggatctcgtcgtgacccatggcgatgcctgcttgccgaatatcatggtggaaaatggccgcttttctggattcatcgactgtggccggctgggtgtggcggaccgctatcaggacatagcgttggctacccgtgatattgctgaagagcttggcggcgaatgggctgaccgcttcctcgtgctttacggtatcgccgctcccgattcgcagcgcatcgccttctatcgccttcttgacgagttcttctgagcgggactctggggttcgcgaaatgaccgaccaagcgacgcccaacctgccatcacgagatttcgattccaccgccgccttctatgaaaggttgggcttcggaatcgttttccgggacgccggctggatgatcctccagcgcggggatctcatgctggagttcttcgcccaccccaacttgtttattgcagcttataatggttacaaataaagcaatagcatcacaaatttcacaaataaagcatttttttcactgcattctagttgtggtttgtccaaactcatcaatgtatcttatcatgtctgtataccgtcgacctctagctagagcttggcgtaatcatggtcatagctgtttcctgtgtgaaattgttatccgctcacaattccacacaacatacgagccggaagcataaagtgtaaagcctggggtgcctaatgagtgagctaactcacattaattgcgttgcgctcactgcccgctttccagtcgggaaacctgtcgtgccagctgcattaatgaatcggccaacgcgcggggagaggcggtttgcgtattgggcgctcttccgcttcctcgctcactgactcgctgcgctcggtcgttcggctgcggcgagcggtatcagctcactcaaaggcggtaatacggttatccacagaatcaggggataacgcaggaaagaacatgtgagcaaaaggccagcaaaaggccaggaaccgtaaaaaggccgcgttgctggcgtttttccataggctccgcccccctgacgagcatcacaaaaatcgacgctcaagtcagaggtggcgaaacccgacaggactataaagataccaggcgtttccccctggaagctccctcgtgcgctctcctgttccgaccctgccgcttaccggatacctgtccgcctttctcccttcgggaagcgtggcgctttctcaatgctcacgctgtaggtatctcagttcggtgtaggtcgttcgctccaagctgggctgtgtgcacgaaccccccgttcagcccgaccgctgcgccttatccggtaactatcgtcttgagtccaacccggtaagacacgacttatcgccactggcagcagccactggtaacaggattagcagagcgaggtatgtaggcggtgctacagagttcttgaagtggtggcctaactacggctacactagaaggacagtatttggtatctgcgctctgctgaagccagttaccttcggaaaaagagttggtagctcttgatccggcaaacaaaccaccgctggtagcggtggtttttttgtttgcaagcagcagattacgcgcagaaaaaaaggatctcaagaagatcctttgatcttttctacggggtctgacgctcagtggaacgaaaactcacgttaagggattttggtcatgagattatcaaaaaggatcttcacctagatccttttaaattaaaaatgaagttttaaatcaatctaaagtatatatgagtaaacttggtctgacagttaccaatgcttaatcagtgaggcacctatctcagcgatctgtctatttcgttcatccatagttgcctgactccccgtcgtgtagataactacgatacgggagggcttaccatctggccccagtgctgcaatgataccgcgagacccacgctcaccggctccagatttatcagcaataaaccagccagccggaagggccgagcgcagaagtggtcctgcaactttatccgcctccatccagtctattaattgttgccgggaagctagagtaagtagttcgccagttaatagtttgcgcaacgttgttgccattgctacaggcatcgtggtgtcacgctcgtcgtttggtatggcttcattcagctccggttcccaacgatcaaggcgagttacatgatcccccatgttgtgcaaaaaagcggttagctccttcggtcctccgatcgttgtcagaagtaagttggccgcagtgttatcactcatggttatggcagcactgcataattctcttactgtcatgccatccgtaagatgcttttctgtgactggtgagtactcaaccaagtcattctgagaatagtgtatgcggcgaccgagttgctcttgcccggcgtcaatacgggataataccgcgccacatagcagaactttaaaagtgctcatcattggaaaacgttcttcggggcgaaaactctcaaggatcttaccgctgttgagatccagttcgatgtaacccactcgtgcacccaactgatcttcagcatcttttactttcaccagcgtttctgggtgagcaaaaacaggaaggcaaaatgccgcaaaaaagggaataagggcgacacggaaatgttgaatactcatactcttcctttttcaatattattgaagcatttatcagggttattgtctcatgagcggatacatatttgaatgtatttagaaaaataaacaaataggggttccgcgcacatttccccgaaaagtgccacctgacgtcgacggatcgggagatctcccgatcccctatggtcgactctcagtacaatctgctctgatgccgcatagttaagccagtatctgctccctgcttgtgtgttggaggtcgctgagtagtgcgcgagcaaaatttaagctacaacaaggcaaggcttgaccgacaattgcatgaagaatctgcttagg

SEQ ID NO: 5 - protein, 450 aa, Artificial sequence
  Heavy-chain of trastuzumab
EVQLVESGGGLVQPGGSLRLSCAASGFNIKDTYIHWVRQAPGKGLEWVARIYPTNGYTRYADSVKGRFTISADTSKNTAYLQMNSLRAEDTAVYYCSRWGGDGFYAMDYWGQGTLVTVSSASTKGPSVFPLAPSSKSTSGGTAALGCLVKDYFPEPVTVSWNSGALTSGVHTFPAVLQSSGLYSLSSVVTVPSSSLGTQTYICNVNHKPSNTKVDKKVEPKSCDKTHTCPPCPAPELLGGPSVFLFPPKPKDTLMISRTPEVTCVVVDVSHEDPEVKFNWYVDGVEVHNAKTKPREEQYNSTYRVVSVLTVLHQDWLNGKEYKCKVSNKALPAPIEKTISKAKGQPREPQVYTLPPSREEMTKNQVSLTCLVKGFYPSDIAVEWESNGQPENNYKTTPPVLDSDGSFFLYSKLTVDKSRWQQGNVFSCSVMHEALHNHYTQKSLSLSPGK

SEQ ID NO: 6 - protein, 214 aa, Artificial sequence
  Light-chain of trastuzumab
DIQMTQSPSSLSASVGDRVTITCRASQDVNTAVAWYQQKPGKAPKLLIYSASFLYSGVPSRFSGSRSGTDFTLTISSLQPEDFATYYCQQHYTTPPTFGQGTKVEIKRTVAAPSVFIFPPSDEQLKSGTASVVCLLNNFYPREAKVQWKVDNALQSGNSQESVTEQDSKDSTYSLSSTLTLSKADYEKHKVYACEVTHQGLSSPVTKSFNRGEC

SEQ ID NO: 7 - DNA, 8071 bp, Artificial sequence
  Expression plasmid pCDNA3.1-Trastuzumab-UAG142
gacggatcgggagatctcccgatcccctatggtgcactctcagtacaatctgctctgatgccgcatagttaagccagtatctgctccctgcttgtgtgttggaggtcgctgagtagtgcgcgagcaaaatttaagctacaacaaggcaaggcttgaccgacaattgcatgaagaatctgcttagggttaggcgttttgcgctgcttcgcgatgtacgggccagatatacgcgttgacattgattattgactagttattaatagtaatcaattacggggtcattagttcatagcccatatatggagttccgcgttacataacttacggtaaatggcccgcctggctgaccgcccaacgacccccgcccattgacgtcaataatgacgtatgttcccatagtaacgccaatagggactttccattgacgtcaatgggtggagtatttacggtaaactgcccacttggcagtacatcaagtgtatcatatgccaagtacgccccctattgacgtcaatgacggtaaatggcccgcctggcattatgcccagtacatgaccttatgggactttcctacttggcagtacatctacgtattagtcatcgctattaccatggtgatgcggttttggcagtacatcaatgggcgtggatagcggtttgactcacggggatttccaagtctccaccccattgacgtcaatgggagtttgttttggcaccaaaatcaacgggactttccaaaatgtcgtaacaactccgccccattgacgcaaatgggcggtaggcgtgtacggtgggaggtctatataagcagagctctctggctaactagagaacccactgcttactggcttatcgaaattaatacgactcactatagggagacccaagctggctagcgtttaaacttaagcttatgtaccggatgcagctgctgagctgtatcgccctgtctctggccctcgtgaccaacagcgaagtgcagctggtggaaagcggcggaggactggtgcagcctggcggatctctgagactgagctgtgccgccagcggcttcaacatcaaggacacctacatccactgggtgcgccaggcccctggcaagggactggaatgggtggccagaatctaccccaccaacggctacaccagatacgccgacagcgtgaagggccggttcaccatcagcgccgacaccagcaagaacaccgcctacctgcagatgaacagcctgcgggccgaggacaccgccgtgtactactgtagtagatggggaggcgacggcttctacgccatggactattggggccagggcaccctcgtgacagtgtctagtgcgtagaccaaggggccctcggtcttccccctggcaccctcctccaagagcacctctgggggcacagcggccctgggctgcctggtcaaggactacttccccgaaccggtgacggtgtcgtggaactcaggcgccctgaccagcggcgtgcacaccttcccggctgtcctacagtcctcaggactctactccctcagcagcgtggtgaccgtgccctccagcagcttgggcacccagacctacatctgcaacgtgaatcacaagcccagcaacaccaaggtggacaagaaagttgagcccaaatcttgtgacaaaactcacacatgcccaccgtgcccagcacctgaactcctggggggaccgtcagtcttcctcttccccccaaaacccaaggacaccctcatgatctcccggacccctgaggtcacatgcgtggtggtggacgtgagccacgaagaccctgaggtcaagttcaactggtacgtggacggcgtggaggtgcataatgccaagacaaagccgcgggaggagcagtacaacagcacgtaccgtgtggtcagcgtcctcaccgtcctgcaccaggactggctgaatggcaaggagtacaagtgcaaggtctccaacaaagccctcccagcccccatcgagaaaaccatctccaaagccaaagggcagccccgagaaccacaggtgtacaccctgcccccatcccgggatgagctgaccaagaaccaggtcagcctgacctgcctggtcaaaggcttctatcccagcgacatcgccgtggagtgggagagcaatgggcagccggagaacaactacaagaccacgcctcccgtgctggactccgacggctccttcttcctctacagcaagctcaccgtggacaagagcaggtggcagcaggggaacgtcttctcatgctccgtgatgcatgaggctctgcacaaccactacacgcagaagagcctctccctgtctcccggcaagtgataaggccggcccctctccctcccccccccctaacgttactggccgaagccgcttggaataaggccggtgtgcgtttgtctatatgttattttccaccatattgccgtcttttggcaatgtgagggcccggaaacctggccctgtcttcttgacgagcattcctaggggtctttcccctctcgccaaaggaatgcaaggtctgttgaatgtcgtgaaggaagcagttcctctggaagcttcttgaagacaaacaacgtctgtagcgaccctttgcaggcagcggaaccccccacctggcgacaggtgcctctgcggccaaaagccacgtgtataagatacacctgcaaaggcggcacaaccccagtgccacgttgtgagttggatagttgtggaaagagtcaaatggctctcctcaagcgtattcaacaaggggctgaaggatgcccagaaggtaccccattgtatgggatctgatctggggcctcggtacacatgctttacatgtgtttagtcgaggttaaaaaaacgtctaggccccccgaaccacggggacgtggttttcctttgaaaaacacgatgataatatggccacaaccatgtaccgcatgcaactcctgtcttgcattgcactaagtcttgcacttgtcacaaacagtgatatccagatgacccagagccccagcagcctgtctgccagcgtgggcgacagagtgaccatcacctgtagagccagccaggacgtgaacaccgccgtggcctggtatcagcagaagcctggcaaggcccccaagctgctgatctacagcgccagcttcctgtacagcggcgtgcccagcagattcagcggcagcagatccggcaccgacttcaccctgaccatcagctccctgcagcccgaggacttcgccacctactactgccagcagcactacaccaccccccccacatttggccagggcaccaaggtggaaatcaagcgtacggtggctgcaccatctgtcttcatcttcccgccatctgatgagcagttgaaatctggaactgcctctgttgtgtgcctgctgaataacttctaccccagagaagccaaagtgcagtggaaggtggacaacgccctgcagagcggaaacagccaggaaagcgtgacagagcaggattccaaggattccacatacagcctgagcagcacactgacactgtccaaggccgactacgagaagcacaaggtgtacgcctgcgaagtgacacaccagggactgtcctcccctgtgacaaagagcttcaacagaggagaatgctgatgatctagagggcccgtttaaacccgctgatcagcctcgactgtgccttctagttgccagccatctgttgtttgcccctcccccgtgccttccttgaccctggaaggtgccactcccactgtcctttcctaataaaatgaggaaattgcatcgcattgtctgagtaggtgtcattctattctggggggtggggtggggcaggacagcaagggggaggattgggaagacaatagcaggcatgctggggatgcggtgggctctatggcttctgaggcggaaagaaccagctggggctctagggggtatccccacgcgccctgtagcggcgcattaagcgcggcgggtgtggtggttacgcgcagcgtgaccgctacacttgccagcgccctagcgcccgctcctttcgctttcttcccttcctttctcgccacgttcgccggctttccccgtcaagctctaaatcgggggctccctttagggttccgatttagtgctttacggcacctcgaccccaaaaaacttgattagggtgatggttcacgtagtgggccatcgccctgatagacggtttttcgccctttgacgttggagtccacgttctttaatagtggactcttgttccaaactggaacaacactcaaccctatctcggtctattcttttgatttataagggattttgccgatttcggcctattggttaaaaaatgagctgatttaacaaaaatttaacgcgaattaattctgtggaatgtgtgtcagttagggtgtggaaagtccccaggctccccagcaggcagaagtatgcaaagcatgcatctcaattagtcagcaaccaggtgtggaaagtccccaggctccccagcaggcagaagtatgcaaagcatgcatctcaattagtcagcaaccatagtcccgcccctaactccgcccatcccgcccctaactccgcccagttccgcccattctccgccccatggctgactaattttttttatttatgcagaggccgaggccgcctctgcctctgagctattccagaagtagtgaggaggcttttttggaggcctaggcttttgcaaaaagctcccgggagcttgtatatccattttcggatctgatcaagagacaggatgaggatcgtttcgcatgattgaacaagatggattgcacgcaggttctccggccgcttgggtggagaggctattcggctatgactgggcacaacagacaatcggctgctctgatgccgccgtgttccggctgtcagcgcaggggcgcccggttctttttgtcaagaccgacctgtccggtgccctgaatgaactgcaggacgaggcagcgcggctatcgtggctggccacgacgggcgttccttgcgcagctgtgctcgacgttgtcactgaagcgggaagggactggctgctattgggcgaagtgccggggcaggatctcctgtcatctcaccttgctcctgccgagaaagtatccatcatggctgatgcaatgcggcggctgcatacgcttgatccggctacctgcccattcgaccaccaagcgaaacatcgcatcgagcgagcacgtactcggatggaagccggtcttgtcgatcaggatgatctggacgaagagcatcaggggctcgcgccagccgaactgttcgccaggctcaaggcgcgcatgcccgacggcgaggatctcgtcgtgacccatggcgatgcctgcttgccgaatatcatggtggaaaatggccgcttttctggattcatcgactgtggccggctgggtgtggcggaccgctatcaggacatagcgttggctacccgtgatattgctgaagagcttggcggcgaatgggctgaccgcttcctcgtgctttacggtatcgccgctcccgattcgcagcgcatcgccttctatcgccttcttgacgagttcttctgagcgggactctggggttcgaaatgaccgaccaagcgacgcccaacctgccatcacgagatttcgattccaccgccgccttctatgaaaggttgggcttcggaatcgttttccgggacgccggctggatgatcctccagcgcggggatctcatgctggagttcttcgcccaccccaacttgtttattgcagcttataatggttacaaataaagcaatagcatcacaaatttcacaaataaagcatttttttcactgcattctagttgtggtttgtccaaactcatcaatgtatcttatcatgtctgtataccgtcgacctctagctagagcttggcgtaatcatggtcatagctgtttcctgtgtgaaattgttatccgctcacaattccacacaacatacgagccggaagcataaagtgtaaagcctggggtgcctaatgagtgagctaactcacattaattgcgttgcgctcactgcccgctttccagtcgggaaacctgtcgtgccagctgcattaatgaatcggccaacgcgcggggagaggcggtttgcgtattgggcgctcttccgcttcctcgctcactgactcgctgcgctcggtcgttcggctgcggcgagcggtatcagctcactcaaaggcggtaatacggttatccacagaatcaggggataacgcaggaaagaacatgtgagcaaaaggccagcaaaaggccaggaaccgtaaaaaggccgcgttgctggcgtttttccataggctccgcccccctgacgagcatcacaaaaatcgacgctcaagtcagaggtggcgaaacccgacaggactataaagataccaggcgtttccccctggaagctccctcgtgcgctctcctgttccgaccctgccgcttaccggatacctgtccgcctttctcccttcgggaagcgtggcgctttctcatagctcacgctgtaggtatctcagttcggtgtaggtcgttcgctccaagctgggctgtgtgcacgaaccccccgttcagcccgaccgctgcgccttatccggtaactatcgtcttgagtccaacccggtaagacacgacttatcgccactggcagcagccactggtaacaggattagcagagcgaggtatgtaggcggtgctacagagttcttgaagtggtggcctaactacggctacactagaagaacagtatttggtatctgcgctctgctgaagccagttaccttcggaaaaagagttggtagctcttgatccggcaaacaaaccaccgctggtagcggtttttttgtttgcaagcagcagattacgcgcagaaaaaaaggatctcaagaagatcctttgatcttttctacggggtctgacgctcagtggaacgaaaactcacgttaagggattttggtcatgagattatcaaaaaggatcttcacctagatccttttaaattaaaaatgaagttttaaatcaatctaaagtatatatgagtaaacttggtctgacagttaccaatgcttaatcagtgaggcacctatctcagcgatctgtctatttcgttcatccatagttgcctgactccccgtcgtgtagataactacgatacgggagggcttaccatctggccccagtgctgcaatgataccgcgagacccacgctcaccggctccagatttatcagcaataaaccagccagccggaagggccgagcgcagaagtggtcctgcaactttatccgcctccatccagtctattaattgttgccgggaagctagagtaagtagttcgccagttaatagtttgcgcaacgttgttgccattgctacaggcatcgtggtgtcacgctcgtcgtttggtatggcttcattcagctccggttcccaacgatcaaggcgagttacatgatcccccatgttgtgcaaaaaagcggttagctccttcggtcctccgatcgttgtcagaagtaagttggccgcagtgttatcactcatggttatggcagcactgcataattctcttactgtcatgccatccgtaagatgcttttctgtgactggtgagtactcaaccaagtcattctgagaatagtgtatgcggcgaccgagttgctcttgcccggcgtcaatacgggataataccgcgccacatagcagaactttaaaagtgctcatcattggaaaacgttcttcggggcgaaaactctcaaggatcttaccgctgttgagatccagttcgatgtaacccactcgtgcacccaactgatcttcagcatcttttactttcaccagcgtttctgggtgagcaaaaacaggaaggcaaaatgccgcaaaaaagggaataagggcgacacggaaatgttgaatactcatactcttcctttttcaatattattgaagcatttatcagggttattgtctcatgagcggatacatatttgaatgtatttagaaaaataaacaaataggggttccgcgcacatttccccgaaaagtgccacctgacgtc